European Patent Application EP 4 375 278 A1, published May 29, 2024. Title: 물질 특성이 개선된 면역조절아마이드 유도체. Applicant: 주식회사 아이비스바이오. Application KR. The sequence listing filed with the application follows.

SEQUENCE LISTING (10 sequences)

SEQ ID NO: 1 - DNA, 21 bp, synthetic construct
  source 1..21: mol_type = other DNA
cccagggacctctctctaatc

SEQ ID NO: 2 - DNA, 21 bp, synthetic construct
  source 1..21: mol_type = other DNA
atgggctacaggcttgtcact

SEQ ID NO: 3 - DNA, 21 bp, synthetic construct
  source 1..21: mol_type = other DNA
acagatgaagtgctccttcca

SEQ ID NO: 4 - DNA, 21 bp, synthetic construct
  source 1..21: mol_type = other DNA
gtcggagattcgtagctggat

SEQ ID NO: 5 - DNA, 20 bp, synthetic construct
  source 1..20: mol_type = other DNA
ggcactggcagaaaacaacc

SEQ ID NO: 6 - DNA, 21 bp, synthetic construct
  source 1..21: mol_type = other DNA
gcaagtctcctcattgaatcc

SEQ ID NO: 7 - DNA, 20 bp, synthetic construct
  source 1..20: mol_type = other DNA
agagtgattgagagtggacc

SEQ ID NO: 8 - DNA, 19 bp, synthetic construct
  source 1..19: mol_type = other DNA
acttctccacaaccctctg

SEQ ID NO: 9 - DNA, 21 bp, synthetic construct
  source 1..21: mol_type = other DNA
ggatgcagaaggagatcactg

SEQ ID NO: 10 - DNA, 20 bp, synthetic construct
  source 1..20: mol_type = other DNA
cgatccacacggagtacttg